European Patent Specification EP 3 185 893 B1, published July 5, 2023. Title: Vaccine,  pharmaceutical composition, carrier for nucleic acids and for other biologically active substances, use of composition in vaccine manufacturing and use of cationic derivatives of polyprenols PTAI in production of immunomodulating substances. Applicant: Instytut Chemii i Biofizyki PAN Uniwersytet Jagiellonski Instytut Chemii Organicznej PAN. Application PCT/PL2015/0000. The sequence listing filed with the application follows.

SEQUENCE LISTING (1 sequence)

SEQ ID NO: 1 - DNA, 1689 bp, Artificial Sequence
  Nucleotide sequence (K3) encoding H5 hemagglutinin from the H5N1 A/swan/Poland/305-135V08/2006 virus, modified in order to achieve optimal expression in chicken cells (Gallus gallus). In addition to codon changes to optimal codons, a sequence coding 6 aa
atggaaaagattgtgctgctgtttgctatcgtgtccctggtgaaaagcgaccagatttgtatcgggtatcatgccaataactcaaccgaacaggtggatactattatggagaaaaacgtgactgtgacccacgcccaggacatcctggagaagacccataacggcaaactgtgcgatctggacggagtgaagcccctgatcctgcgcgattgcagcgtggctggctggctgctgggaaaccctatgtgcgacgagttcctgaatgtgccagaatggtcctacatcgtggagaaaattaacccagcaaatgatctgtgctaccccggcaacttcaatgactatgaggaactgaagcacctgctgtctaggatcaaccatttcgaaaagatccagatcatccctaagagctcctggagcgatcacgaggcttcttcaggcgtgagtagcgcatgtccataccagggacgctcctctttctttcggaacgtggtgtggctgattaagaaagacaatgcttacccaactatcaaacgcagctataacaataccaaccaggaagatctgctggtgctgtggggaatccaccatcccaacgacgccgctgagcagacacggctgtaccagaatcctaccacatatattagtgtggggacaagcactctgaaccagagactggtgcccaagatcgcaacaaggagcaaagtgaatggccagtccggaagaatggagttcttttggactatcctgaagccaaacgatgccattaatttcgaatctaacggcaacttcatcgcacccgagaacgcctacaagattgtgaagaaaggagactccactatcatgaaatctgagctggaatatgggaactgcaataccaagtgtcagacacctatcggtgcaattaactcaagtatgccctttcacaatatccatcctctgaccattggggagtgccccaagtacgtgaaaagtaaccgcctggtgctggccacaggtctgcggaatagccctcagggggaaggtctgttcggggctatcgcaggttttattgagggcggatggcagggaatggtggatgggtggtacggttatcaccattcaaacgaacagggcagtggatacgcagccgataaggagtcaacacagaaagccattgacggagtgactaacaaggtgaactccatcattaacaaaatgaacacccagttcgaggctgtggggagagagttcaacaatctggagagaaggatcgaaaacctgaataagaaaatggaagatggcttcctggacgtgtggacttacaacgctgagctgctggtgctgatggagaatgaaaggaccctggattttcacgacagcaacgtgaagaatctgtatgataaagtgagactgcagctgagggacaacgcaaaggaactggggaatggttgtttcgagttttaccatagatgcgataacgagtgtatggaatccgtgaggaatggcacatacgactatccacagtattctgaggaagcccgcctgaagcgggaggaaatttctggggtgaaactggagtcaatcggtacctaccagatcctgtctatctactcaacagtggctagctccctggccctggctatcatggtggctggcctgagcctgtggatgtgctctaacggtagcctgcagtgtaggatctgtatttga